European Patent Application EP 4 628 589 A1, published October 8, 2025. Title: A microorganism introduced with exogenous glutamine synthase and method for producing L-tryptophan using the same. Applicant: CJ CheilJedang Corporation. The sequence listing filed with the application follows.

SEQUENCE LISTING (67 sequences)

SEQ ID NO: 1 - protein, 445 aa, Aureibacillus halotolerans
MGSKYTRKDIVKLVEEENVRFIRLQFTDLLGIIKNVEIPVDQLGKALDNKMMFDGSSIEGFVRIEESDMYLYPDLDTFVVFPWTSEKGRVARLICDIYNPDGTPFAGDPRSVLKKVIQEMKDLGFTAFNIGPEPEFFLFKNDEKGEPTLELNDKGGYFDLAPTDLGENCRRDIVLELEDMGFEIEASHHEVAPGQHEIDFKYADAVKACDDIQTFKLVVKTIARKHGLHATFMPKPLFGVNGSGMHANMSLFKGEQNAFFDEKSDLQLSETAKQFIAGILKHAEAFTAITNPTVNSYKRLVPGYEAPCYVAWSSRNRSPLVRIPASRGLSTRIEVRSVDPAANPYLAMAVMLAAGLDGVKNNLTPPAPVDRNIYVMDKEERIENGIADLPATLAQALDTLKRDDIIMAALGEHAAEHFIEAKEIEWDMFRTQVHPWEREQYLTLY

SEQ ID NO: 2 - DNA, 1338 bp, Aureibacillus halotolerans
  source 1..1338: mol_type = genomic DNA
atgggttctaagtacacgagaaaagacatcgtaaagcttgttgaggaagagaacgtacgttttatacgtttgcagtttacagatttgctaggaattataaaaaacgttgagatccctgttgatcaattgggtaaagccttagacaacaaaatgatgtttgacggctcatccattgaagggtttgttcgtatcgaggaatcagacatgtatctctatccagatctagatacctttgttgtattcccatggacgagcgaaaaaggtcgcgtagctcgtttaatttgtgatatttacaatccggatggcacaccgttcgcaggtgatccaagaagcgtacttaaaaaagtcattcaagaaatgaaagatctcggctttactgcctttaatatcggaccagagcctgagtttttccttttcaaaaatgatgaaaaaggtgagcctacgcttgagttgaatgacaaaggcggctattttgacttagcaccaacggatctaggtgaaaattgtcgacgtgatatcgtgcttgagcttgaagacatgggctttgaaattgaagcatcacaccatgaagtcgctcctggtcaacacgaaatcgactttaaatatgcagacgctgtaaaagcgtgtgacgacattcaaacgtttaagcttgttgttaaaacaattgcacgtaagcacggcttgcatgcgacgtttatgccaaaaccattgtttggtgtgaatggttctggtatgcacgcaaacatgagcttgtttaaaggtgagcaaaacgcgttttttgacgaaaaatcagaccttcaattaagcgaaacagcaaagcaatttattgctggcattctgaagcatgctgaagcatttacagccattacgaacccaacagtaaactcatacaagcgtttagtgcctggctacgaagccccatgttacgttgcatggtcttctcgtaaccgttcaccactcgtacgtatcccagcttctcgtggcttgagcacacgtatcgaagtgcgttcggttgacccagctgcgaacccttacttggccatggctgtaatgcttgctgctggacttgacggtgtgaaaaacaacttaacaccaccagcaccagtagatcgcaacatctacgtgatggacaaggaagagcgtattgaaaacggcattgctgatcttccagcaacgcttgcccaagcgcttgacactcttaagcgtgacgatatcatcatggcagcacttggtgagcacgctgcagaacactttatcgaagcaaaagaaatcgaatgggacatgttccgcacacaagttcacccttgggagcgcgagcagtaccttaccctttactaa

SEQ ID NO: 3 - protein, 444 aa, Caryophanon tenue
MGKYTKDDIHRLVKEQEVKFIRLQFTDILGTIKNVEIPVSQLDKALDNKMMFDGSSIEGFVRIEESDMYLFPDYDTFMIFPWTAEKGKVARFICDIARPDGTPFEGDPRSNLKRVLKEMEDLGFTDFNLGPEPEFFLFKLDAKGEPTLEVNDHGGYFDLAPTDLGENCRRDIVLELEEMGFEIEASHHEVAPGQHEIDFKYADAIQACDNIQTFKLVVKTIARKHGLHATFMPKPLFGEAGSGMHFNVSLFKGKENAFYDDSTELGLSETAMQFMAGVLNHVKGFTAVINPTINSYKRLVPGYEAPCYVAWSAQNRSPLIRIPSSRGVSTRVEVRSVDPSANPYLAMAVILEAGLEGIRQQATPPAAINRNIYVMSETERKANGIDNLPASLEHALQLLAEDEVAKKALGEHIYANFREAKEIECEMFRTQVHQWERDQYLKMY

SEQ ID NO: 4 - DNA, 1335 bp, Caryophanon tenue
  source 1..1335: mol_type = genomic DNA
atgggtaaatacacaaaagacgatatccatcgtttagtcaaagaacaagaagtaaaattcatccgtttacagtttactgatattttaggaacgattaaaaacgttgaaattccagtaagccagttagacaaagcgttagacaacaaaatgatgttcgatggttcatcaatcgaaggtttcgttcgtattgaagaatcagatatgtacttattccctgattacgatacatttatgattttcccttggacagctgaaaaaggcaaagtagcacgttttatttgtgacattgctcgtccagacggaacaccttttgagggggacccacgttcgaacttaaagcgcgtattaaaagaaatggaagatctagggttcacagactttaacttagggcctgagccagaattcttcttattcaaattagacgctaaaggcgaaccaactcttgaggtaaacgaccacggtggttacttcgacttagcaccaacagatttaggtgaaaactgtcgtcgtgatatcgtattagagcttgaagaaatgggctttgaaatcgaagcatcacaccatgaagtagcaccaggtcagcacgaaatcgactttaaatatgcagatgcaattcaagcatgtgataatatccaaacatttaaattagttgtaaaaacaatcgcacgtaaacacggtttacacgctacatttatgccaaagccattattcggtgaagctggttcaggcatgcactttaacgtatcattatttaaaggcaaagaaaatgctttctatgatgactcaacagagctaggcttatcagaaacagcaatgcaatttatggcgggagtgttaaaccacgtaaaaggtttcacagcggttattaacccaacaattaactcatacaaacgtttagtaccaggttacgaagcaccatgttacgtagcatggtcagcacaaaaccgttcaccattaattcgtattccatcgtctcgtggtgtatcaacacgcgtagaagtacgttcagtagacccatctgcaaacccatacttagcgatggcggtgattttagaagctggtctagaaggtattcgtcaacaagcgacaccaccagcagcaattaaccgcaacatttatgtgatgagtgaaacagagcgtaaagcaaacggtattgataatttaccagcttcattagaacatgcattacaattacttgcagaagatgaagtagcgaaaaaagcattaggtgaacacatctatgcaaacttccgagaagcaaaagaaattgagtgtgaaatgttccgtacacaagtacatcaatgggaacgtgaccaatatttaaaaatgtattaa

SEQ ID NO: 5 - protein, 444 aa, Peribacillus simplex
MAKFTREDITRLAKEENVKYIRLQFTDILGTIKNVEIPVSQLEKALDNKMMFDGSSIEGFVRIEESDMYLYPDLNTWVIFPWTSEKGKVARLICDIYNTDGTPFDGDPRANLKRVLAEAREMGFTDFNLGPEPEFFLFKLDAAGEPTLELNDKGGYFDLAPTDLGENCRRDIVLELEEMGFEIEASHHEVAPGQHEIDFKYADAISACDNIQTFKLVVKTIARKHGLHATFMPKPLFGVNGSGMHCNVSLFKGNENAFYDTKGKLELSKTAEQFIAGIIKHAPSFTAVTNPTVNSYKRLVPGYEAPCYVAWSAKNRSPLIRIPASRGVSTRVEVRSVDPAANPYLALAVLLKAGLDGIKNDLTPPAPVDRNIYVMNKEEREEVGIVDLPATLYAALETLKSDEVIKEALGEHLLEHFIEAKEIEWDMFRTQVHPWEREQYMSMY

SEQ ID NO: 6 - DNA, 1335 bp, Peribacillus simplex
  source 1..1335: mol_type = genomic DNA
atggcaaagttcacacgtgaagacatcactcgtttagcgaaagaagaaaatgttaagtacattcgtttacaatttactgatattttagggacaattaaaaacgttgaaatcccagtcagtcaattagaaaaagcacttgataataaaatgatgtttgacggatcttccattgaaggcttcgtacgtatcgaagagtctgatatgtacctatatcctgatttaaatacatgggttatcttcccttggacttccgaaaaaggtaaagtcgcacgtttgatctgtgatatttacaatacggatggaacaccttttgatggagatccacgtgcaaacctaaaacgtgttcttgcagaagcaagagaaatgggcttcacagatttcaatcttggacctgaacctgaattcttcctatttaaactggatgcagcaggcgagccgactttagaattgaacgacaaaggcggatactttgaccttgcacctactgacctaggagaaaactgccgtcgtgatatcgttcttgagcttgaagaaatgggatttgaaatcgaagcatcccaccatgaagtagctccaggacaacatgaaattgactttaaatatgcagatgcaatctcagcttgtgataacatccaaacatttaaattggttgttaaaacaattgcccgtaaacatggtttacacgcaacattcatgccaaaaccattgttcggtgttaacggatctggtatgcactgtaacgtttctctattcaaaggaaacgaaaacgcattttatgatacaaaaggtaaattggaattaagtaaaacagctgagcaatttatcgcaggtatcattaagcatgctccaagcttcactgcggtaacaaacccaactgttaactcatacaaacgtctagttcctggttacgaagctccttgttatgttgcatggtccgctaaaaaccgtagcccattaatccgtatcccagcttcacgtggagtaagtactcgcgtagaggtacgtagtgtcgatccagcagcaaacccatacttggcacttgcagttctgctgaaagctggtcttgacggtatcaagaacgacttgactcctccagctccagttgaccgcaacatctatgttatgaataaagaagagcgtgaagaagtaggtatcgttgatctaccagctactttgtatgctgcattggaaacattaaaatctgatgaagtaatcaaagaagcattaggtgaacatttacttgaacacttcatcgaagcaaaagaaatcgagtgggatatgttccgcacacaagttcacccatgggaacgcgaacaatatatgtcaatgtattaa

SEQ ID NO: 7 - protein, 444 aa, Carnobacterium divergens
MPEFTREQITKIAKEEDVRFLRLMFTDIMGIIKNVEVPISQLEKVLDNKMMFDGSSIEGFVRIEESDMYLRPDLTSWLIFPWGTGKGKIARLICDIYNPDGTPFAGDPRSNLKRVLKEMEEFGFTSFNLGPEPEFFLFKLDEKGEPTLELNDKGGYFDFAPTDLGENCRREIVLQLEEMGFEIEASHHEVAPGQHEIDWKYANAIEACDYIQTFKLVVKTVARQHGLHATFMPKPLFGVNGSGMHFNMSLFTEDGNAFYDEEGDMQLSETARQFLAGVLSHARAYTAICNPTVNSYKRLVPGYEAPVYVAWSGRNRSPLIRVPESRGLSTRIELRSVDPTANPYLAMAVLLKSGLDGIRNEMVAPAPVDRNIYVMTEEERHERGINDLPSTLHNAIKYLRQDEVVKAGLGSHIYNNFVEAKRLEWAAFRQQVSEWEREQYLELY

SEQ ID NO: 8 - DNA, 1335 bp, Carnobacterium divergens
  source 1..1335: mol_type = genomic DNA
atgccagaatttacaagagaacaaatcaccaagattgcgaaagaggaagatgtacgttttttacgtttaatgtttacagatattatgggaattattaaaaatgttgaagttccaatcagtcagctggaaaaagtattagacaacaaaatgatgtttgacggatcttcaattgaaggttttgtacgaattgaagaaagtgatatgtatttacgcccagatttaacttcttggttgatttttccttggggaactggaaaaggcaaaattgcgcgtttaatctgtgatatctacaatcctgatgggactccatttgctggcgatcctcgtagcaatttaaaacgagtattaaaagaaatggaagaatttggctttacctctttcaacttaggaccagagcctgaatttttcttattcaaactagatgaaaaaggtgaaccaactcttgagttaaatgataaaggaggctatttcgacttcgcgccaacagacttaggtgaaaattgtcgtcgtgaaattgtcttacaattagaagaaatgggctttgaaatcgaagctagccaccatgaagtagcgccaggtcaacatgaaatcgattggaaatatgcaaatgcaattgaagcatgtgattatatccaaacctttaaacttgttgtcaaaactgtagctcgtcaacatggacttcacgcaacctttatgccaaaaccgttatttggtgtaaatggatcagggatgcatttcaatatgtctttatttacagaagacggcaatgccttttatgatgaagaaggcgatatgcaattaagtgaaacagctcgtcagttcttagcaggtgttttaagtcatgcaagagcctacactgctatttgtaacccgacagtgaattcatacaaacgtttagtacctggctatgaagcgccagtttatgtagcatggagtggacgtaatcgttcaccgttaattcgtgttccagaatctcgtggcttatcaacaagaatcgagctacgcagtgttgacccaacagcaaatccatatttagctatggctgttttattaaaatctggattagatggaattagaaatgaaatggtagcaccagctcccgttgatcggaatatttatgtgatgaccgaagaagaacgtcacgaacgtggcattaatgatcttccatcaacgctccacaatgcgattaaatacttgcgacaagatgaagttgtgaaagctggtttaggttctcatatctacaataattttgttgaagccaaacgtttagagtgggcggcgttccgtcaacaagtttcagaatgggaaagagaacaatatttagagttatactaa

SEQ ID NO: 9 - protein, 445 aa, Bacillus gobiensis
MAKYTREDIVKLVNEENVKYIRLQFTDILGTIKNVEIPVSQLEKALDNKCMFDGSSIEGFVRIEESDMYLYPDLNTFVIFPWTAEKGKVARFICDIYSPDGTPFEGDPRNNLKRILKEMEELGFTDFNLGPEPEFFLFKLDEKGDPTLELNDKGGYFDLAPTDLGENCRRDIVLELEEMGFEIEASHHEVAPGQHEIDFKYAGALRSCDDIQTFKLVVKTIARKHGLHATFMPKPLFGVNGSGMHCNLSLFKEGGVNAFYDENGELQLSETARHFIAGIIKHATSFTAVTNPTVNSYKRLVPGYEAPCYVAWSARNRSPLIRIPASRGISTRVEVRSVDPAANPYLAMSVLLAAGLDGIKNQLSAPAPIDRNIYVMSKEERIESGIVDLPSTLALALEELKSNQVMVDALGEHLFAHFIEAKEIEWDMFRTQVHPWERDQYLTQF

SEQ ID NO: 10 - DNA, 1338 bp, Bacillus gobiensis
  source 1..1338: mol_type = genomic DNA
atggcaaagtatactagagaagatattgtcaaattagtaaacgaggaaaacgtaaagtatatccgtctgcaatttacagacattttaggaacaattaaaaacgtagaaattcctgttagccagcttgaaaaagcgcttgacaacaagtgcatgtttgatggttcttctatcgaagggttcgtaagaattgaagaatctgacatgtatttatacccggatttaaatacttttgtcattttcccttggactgctgaaaaaggtaaagtagcccgttttatttgtgacatttacagcccggatggtacaccgtttgaaggggatccgcgtaacaacctaaaacgaatcttgaaagaaatggaagaattaggattcactgatttcaacttagggcctgagcctgaattcttcttgttcaaattagatgaaaaaggagacccgacactagagcttaacgataaaggcggatatttcgaccttgctccaactgaccttggtgaaaactgccgtcgtgatatcgttcttgagcttgaagaaatgggatttgaaatcgaagcgtctcaccatgaagttgctcctggtcagcacgaaattgattttaaatatgccggtgcccttcgttcatgcgatgacatccaaacgtttaaacttgttgttaaaacaattgcccgcaaacacggtttgcatgcgacattcatgcctaaaccattgtttggcgtaaacggatctggtatgcactgtaacctttccctatttaaagagggaggagtaaacgcattttatgatgaaaatggagaattgcaattaagcgaaactgctagacactttatcgctggaattattaagcatgctacaagctttacagcagtaacaaacccaacggtaaactcttacaaacgtttggttcctggatacgaagctccatgttatgtcgcttggagtgcacgtaacagaagcccgttaattcgtatcccagcttctcgcggtataagtactcgcgtagaagttcgcagcgtagatccagctgctaacccatacttggcaatgagtgttcttttagctgctggtttagacggaattaaaaatcaattatctgctccggcaccaattgaccgaaacatctatgtcatgagcaaagaagagcgtattgaaagcggcatcgttgatttaccatcaactttggcacttgccttagaagagctaaaatccaatcaagttatggtcgatgcgcttggtgagcatttattcgcacacttcattgaagcaaaagaaatcgagtgggatatgttccgcacacaagtacatccttgggaacgcgatcaatatttaactcagttttaa

SEQ ID NO: 11 - protein, 444 aa, Carnobacterium inhibens
MKKFTRKEIEISAKEENVRYLRLMFTDIDGIIKNVEVPISQLEKVMDNKMMFDGSSIDGFVRIEESDMILCPDLSTWLIFPWESENGKIARLICDIYNPDGTPFAGDPRNNLKRVLKQMEEQGFTEFNLGPEPEFFLFKLDENGKPTTELNDNGGYFDFAPTDLGENCRRDIVLQLEELGFEIEASHHETAPGQHEIDWKYASAIEACDNIQTFKLIVKTVARKHGLHATFMPKPMFGVSGSGMHFNMSLFNNQGNVLCNEEDELGLSKTAYHFLAGILDHALGYTAICNPTVNSYKRLIPGYEAPVYIAWSARNRSPLVRIPSSRGVSTRIELRSVDPSANPYLAVATLLYSGLDGVKKEMEVPKPIDRNIYRMSSEERYKKGIKDLPSTLHNAVKYLQEDKVVQEALGEHIYRSFVSAKHVEWAAYREQVSEWEKEKYLTLY

SEQ ID NO: 12 - DNA, 1335 bp, Carnobacterium inhibens
  source 1..1335: mol_type = genomic DNA
atgaaaaaatttacaaggaaagaaatcgaaataagtgcaaaagaagaaaatgttcggtatttacgattgatgtttacggatatagatggaatcattaaaaatgttgaggtgcctattagtcaactagaaaaagtcatggacaataaaatgatgtttgatggctcttccattgatggttttgtaagaattgaagaaagcgacatgattttgtgcccagatttatcaacgtggttaattttcccttgggaatctgaaaacggaaaaattgctcgtttgatttgtgatatttataatccggacggtacaccatttgctggagatcctagaaacaacttgaagcgtgttctaaaacaaatggaagaacaaggctttacagagtttaatttaggacccgaacccgaatttttcttatttaaattagacgaaaatggaaaaccaacgactgaattaaatgataatggcgggtatttcgattttgctccaacggatttaggcgaaaactgtcgccgtgatattgtgttgcaactagaagaattaggttttgaaattgaagctagtcatcatgaaacagctcccggtcagcatgagatagactggaaatatgcaagtgccatagaagcatgtgacaatatccaaacgtttaaactaatcgtaaaaacagttgcccgcaaacatggtttgcatgcgacattcatgcctaaaccaatgtttggtgtaagtggttctggaatgcattttaacatgtctttatttaacaatcagggcaatgttctttgtaatgaagaagatgaacttggtttaagtaaaacggcttatcatttcttagcaggtatattggatcatgctttaggatatacggctatctgtaatccgactgtaaactcttataaacgattgattccaggatacgaagcacctgtttatatcgcatggagtgctcgtaatcgctcaccacttgtgcgtattccaagctcaagaggagtttctactcgtattgaattgcggagtgttgatcctagtgctaatccttatttagccgttgcaacattgttgtattcaggactagatggagtgaaaaaagaaatggaagtacctaaaccaatagatcgcaatatctatcgtatgtcttcagaagaacgatacaaaaaaggcatcaaagatcttccatctactttgcataatgctgttaaatacttgcaagaagataaagtcgttcaagaagctttgggtgaacatatctatagaagttttgtcagtgctaaacatgtagagtgggctgcttatcgtgaacaagtttctgaatgggaaaaagaaaaatatctaaccttatattaa

SEQ ID NO: 13 - protein, 446 aa, Carnobacterium iners
MKNFTREEIVTSAKENNVRFLRLMFTDIDGTVKNVEVPISQLTKALNNEMMFDGSSIDGFVRIEESDMFLYPDLGTWLIFPWEIGNGKGSVARLICDIYNADDTPFSGDPRTNLKRALKEMEKMGFKEFNLGPEPEFFLFKLDKNGKPTLELNDNGGYFDFAPTDLGENCRREIVLHLEDLGFEIEASHHETAPGQHEIDWKYADALEACDNIQTFKLIVKTVAREHGLHATFMPKPLEGVSGSGMHFNMSLFNENGNAFYDESDKLGLSKTAYQFLAGIIDHALAYTAICNPTVNSYKRLIPGYEAPVYVAWSARNRSPLIRVPSSRGMSTRFELRSVDPSANPYLALAVLLRSGLDGIKNEMVPAEPIDRNIYRMTTEERHEKGIIDLPSTLHNALKYLGKDEIVKDALGPHIYNSFVTSKKVEWAAYREQVSEWEQEKYMTLY

SEQ ID NO: 14 - DNA, 1341 bp, Carnobacterium iners
  source 1..1341: mol_type = genomic DNA
atgaaaaattttactagagaagaaatcgtaacaagtgcaaaagaaaataatgttcgttttttacgtttaatgtttactgatattgatggaacggttaagaacgttgaagtacctattagccagttaactaaggcgttaaataatgaaatgatgtttgacggttcttcaattgatggttttgttcgaattgaagaaagcgatatgttcttgtatccagatttaggtacatggttaatttttccttgggaaattggtaatggaaaaggcagtgttgctcgtttgatttgcgatatttataacgctgatgatacgccattttctggtgacccacgaacaaatttaaaacgcgccttaaaagaaatggaaaaaatgggctttaaagaatttaatttaggacctgaacctgaatttttcttatttaaactcgataaaaatgggaaaccaacattagaactaaatgataacggtgggtactttgattttgctccaacagacttaggtgaaaattgccgacgtgaaattgtattacatttagaagatttaggtttcgaaattgaggcaagtcatcacgaaacagctccaggacaacatgaaattgactggaaatacgcagatgctcttgaagcatgtgataacattcaaacttttaaattaatcgttaaaacagtagctcgtgaacatggcctacacgctacatttatgccaaaacctttagaaggtgtaagtggctctggtatgcactttaatatgtctttatttaatgaaaatggcaatgctttttacgatgagtcagataaattaggacttagtaaaacagcgtatcaatttttagctggaataatcgatcacgctttagcttatacagcaatttgtaacccgactgtcaattcttataagcgactaattccaggctatgaagctcccgtttatgtggcttggagcgcacgcaatcgttcgcctttaattcgcgtaccaagttctcgtggaatgtctacacgctttgaattacgtagtgttgatcctagtgcaaatccatatcttgctttagctgttttattgagatcaggtttggatggaatcaaaaacgaaatggttccagcagagcctatcgaccgtaatatttaccgtatgacaactgaagaaagacacgaaaaaggaatcattgacttgccatctactttacacaatgctttgaagtatttaggtaaggatgagatagtaaaagatgctcttggacctcatatctataatagttttgtaacatccaaaaaagtagagtgggcagcttaccgcgaacaagtttctgagtgggaacaagaaaagtatatgactctttattaa

SEQ ID NO: 15 - protein, 448 aa, Lactiplantibacillus paraplantarum
MAKQSYSKDDIRRIVKEENVNFLRLMFTDLFGTIKNVEVPVSQLDKLLDNKLMFDGSSIDGFVRIEESDMYLYPDLSTWLIMPWNTEHGKIARIICEVYTADRKPFEGDPRNNLIRVLNDMREAGYTSFNCGTEPEFFLFKMNEKGEPTTELNDKGSYFDLSPMDLGENCRRDIALELERLGFNVEASHHEVAPGQHEIDFKYADALSAADHIQTFKLVVKTIARKYNLWATFMPKPLNGVNGSGMHVNMSLFHDQGNAFYDANDKSGLELSSDAYHFLGGLMKHARSYTAVTNPTVNSYKRLVPGYEAPVYVAWSASNRSPMIRIPSARGLSTRLELRSVDASTNPYLAFAAVLEAGLDGIKNGIEPPKSVDRNIYVMDEDERSAAGIADLPSTLHNALKEFQTDPTMKKALGPHIYQSFLEAKRLEWASYRQQVSEWERDQYMELY

SEQ ID NO: 16 - DNA, 1347 bp, Lactiplantibacillus paraplantarum
  source 1..1347: mol_type = genomic DNA
atggcaaaacagtcctattcaaaagacgatatccgccgcatcgtcaaagaagaaaacgttaattttttgcggttaatgtttactgatttatttggcacaattaagaacgttgaagttccggtttcacaactcgacaaacttctggataacaagttgatgtttgatggttcatccatcgatgggtttgttcggatcgaagaaagtgacatgtacctgtatcctgacttatcaacttggttgattatgccttggaatacggaacatggaaaaattgcacggatcatctgtgaagtttacaccgctgaccgtaagccgtttgaaggtgacccacggaacaatttgattcgtgtcttgaatgatatgcgggaagcaggttatacgtcatttaactgtgggactgaacctgaattcttcttatttaaaatgaatgaaaagggcgaaccaacgactgaattgaacgataaggggagttactttgacttatcgccaatggacttaggtgaaaattgtcgtcgggatattgcacttgaactcgaacggcttggctttaacgttgaagccagtcaccatgaagttgcacctggccaacatgaaattgactttaagtacgcggatgccttatctgcagccgatcatattcaaacattcaagttggtcgttaagaccatcgcacggaaatacaacttgtgggcaaccttcatgcctaagccgttaaacggtgttaatggttctgggatgcatgtgaacatgtccttgttccatgatcaagggaatgctttttacgatgctaatgacaagagtgggttagaattgtcatccgatgcttaccatttcttaggcggtctgatgaagcatgcacgttcttacacggctgttacgaatccaacggtcaactcatacaaacggttggttccaggatacgaagcaccagtgtacgtggcttggtcagcctctaaccggtcaccaatgattcgaattccaagtgcacgcggcttatcaacacgtcttgaattacggagtgtggatgcatcaactaatccatatttagcctttgcagcagtgctggaagctggcttagatggtatcaagaatggcatcgaaccaccaaagagtgttgatcgtaacatttatgtcatggatgaagatgaacgttcagcagctggtatcgctgacttgccatcaacgttacacaacgctctgaaagaattccagacagatccaacaatgaaaaaagcgttggggccacatatttatcagagtttcttggaagctaaacggctagaatgggcatcataccgtcagcaagttagcgaatgggaacgtgatcagtacatggaactgtattaa

SEQ ID NO: 17 - protein, 473 aa, Sulfolobus acidocaldarius
MPGLPKNEHEALEFLKSNNIKWVDLQFTDLLGKLQHITIPSNEFDESSFKVGFGKLDGSSIKGFTSIYESDMVLLPIPQTMTLIPWMQGVARVLTKVFWGGGKGRFERDPRGIAEEAEKYQSEQGYVSYFGPELEFFVFDKVEVDASLPQSGTGYKIHSREAPWSKNGGYVIRYKEGYYPASPVDQLMDIRLEIISTLVDYFGFTIEAAHHEVATAGQGEIDFRFSTLADTADKVQVLKYVTKNIASKRGMIATFMPKPFFGDNGSGMHTHFSLWTKDGKNLMYDPNDEYAELSQIGRYIIGGLLEHGRALSAIVAPTTNSYRRLVPGYEAPVYLVWSKSNRSAAIRIPAYYKGMEKAKRLEYRPPDPSSNPYLVFSAILMAGLDGIRRKLDPGDPVDENIYHMSEEKKRSLKIRELPGSLDEALNELESDNEFLKPVFNSSILQAYLDLKKEEAKMMQLYPHPMEIYQYLDS

SEQ ID NO: 18 - DNA, 1422 bp, Sulfolobus acidocaldarius
  source 1..1422: mol_type = genomic DNA
atgccaggacttccaaaaaatgaacatgaagcactagagtttttgaaaagtaataatataaaatgggttgatttacaatttacagatctcctaggtaaattgcaacatataacaataccatcaaatgaatttgatgaaagctcgtttaaggttggattcggtaagttagacggaagcagcataaagggattcaccagtatttatgaaagcgatatggtattattaccaatacctcaaacaatgacactaataccttggatgcaaggtgtcgcaagagtactgactaaggtattctggggaggtggaaaaggtagatttgagagagatccaagagggatagccgaagaggcagaaaaataccagagcgaacaagggtatgtaagttatttcggaccggaactagaatttttcgtgttcgataaagtagaggtagacgcatcattacctcaaagcggaacaggatataaaatacattccagagaagcaccatggtctaagaatggcggatatgtaataaggtataaagaaggatactatcctgcatcaccagttgatcaattaatggatatacgcttggaaattataagtactttagtagactactttgggtttacaatagaagcagctcatcatgaagtagcaacagcaggtcaaggtgagatagatttcagattctccacattagctgatactgcagataaagtacaggttcttaaatatgtaacaaagaacattgcaagtaaacgtggtatgatagcgacatttatgccaaaaccattcttcggagacaacggtagtggtatgcatactcactttagtttgtggacaaaagatgggaaaaatctaatgtatgatcctaatgatgaatatgcagaattaagccaaataggtagatacattataggcggtctcttagaacatggcagagcattaagcgcaatagtcgcaccaaccactaatagttatagacgtttagtgccagggtatgaagcccctgtatacttggtttggagtaaatctaacagaagtgctgcaataagaattccagcctattacaagggaatggaaaaagctaaaaggttagaatacagaccacctgacccttcatctaatccctaccttgtattctctgcaatacttatggcaggtttagatggaatcagaagaaaactagacccaggtgatccagtggacgaaaacatatatcatatgagtgaagagaagaaaaggagcctgaaaataagagaattaccaggatcattagatgaagctttgaatgagttagagagtgataatgaattcctgaagccagtattcaactcttcaatattacaagcatatctagacctaaagaaagaagaagcaaaaatgatgcaactatatccacatcctatggaaatatatcagtatctagattcttaa

SEQ ID NO: 19 - protein, 443 aa, Petroclostridium xylanilyticum
MPNYTREDVIRMVKEQDVKFIRLQFTDIFGTLKNVAITSSQLEKALNNQCMFDGSSIEGFVRIEESDMYLRPDPNTFAIFPWRPQPGRVARLICDVYNPDGTPFEGDPRYILKKVIKEAKDMGYTFNVGPECEFFLFLTDENGDPTTITHDNAGYFDLGPIDLGENARRDMCLMLEEMGFEIEASHHEVARGQHEIDFKYAEGLTTADNIMTFKLVVKMMAQRHGLHATFMPKPIFGINGSGMHTNMSLSKDGKNAFYDPDDQLGLSEIAYNFIAGILKHIKGMAAVTNPIVNSYKRLVPGYEAPVYIAWSAKNRSPLIRIPAARGASTRIEMRNPDPACNPYLALAVSLAAGLDGIKNGLKPPASVEKNIYHMDEAARKEHGIESLPGSLYEAIIEMQNDELVKKTLGPHAFERYVEAKLIEWNDYRTKVHQWEIDQYLTRY

SEQ ID NO: 20 - DNA, 1332 bp, Petroclostridium xylanilyticum
  source 1..1332: mol_type = genomic DNA
atgcctaactataccagggaagatgtaataaggatggtaaaagagcaggatgttaaattcataaggcttcagtttaccgatatttttggaacgcttaagaatgttgctatcacttccagtcaattagagaaagcattaaataatcaatgcatgtttgatggttcttccatagaaggatttgtaagaatcgaagaatcggatatgtacttgagacctgaccccaatacttttgcaatatttccatggcggccacagccggggagagtggcaagactgatatgcgacgtatataacccggatggaacaccttttgaaggggatccaagatacattctcaaaaaagttattaaagaagcaaaagatatgggatatacctttaacgttgggccggaatgtgaattctttttattccttactgacgagaacggagatcctaccactattacccatgataatgccgggtactttgatttaggacctattgaccttggagaaaatgccagaagagatatgtgcctgatgcttgaagaaatgggatttgaaatagaagcctcccaccatgaagttgcaagaggccagcatgagattgattttaagtatgctgaaggattaactacagcagataatattatgacttttaagctagtagtaaaaatgatggcccaaaggcatggattacatgcaacttttatgcctaagcctatttttggaatcaatggttccgggatgcataccaatatgtccctttccaaggatggtaaaaacgccttttacgacccggatgatcaattaggccttagtgaaattgcgtacaactttattgcaggcatattaaagcatataaaaggaatggctgccgttaccaatcctattgttaactcatataaaagattggtaccgggctatgaagcgccggtatatattgcctggtctgctaaaaataggagcccattgatacgtattcctgcagcaagaggagcaagcacaagaatagaaatgaggaatccagatccggcttgtaacccgtatcttgcccttgcagtttcgttagcagccgggttggatggaataaagaatgggttaaagcctccggcgagtgttgaaaaaaatatttaccacatggatgaagcagcaagaaaagaacatggcattgaaagtttgccgggcagcctgtatgaggcaataatagaaatgcaaaatgatgagttagtcaaaaagactcttgggcctcatgcatttgaacgatatgttgaagctaagctgattgaatggaatgattacaggacaaaggttcatcaatgggaaatcgaccagtatctcaccagatattaa

SEQ ID NO: 21 - protein, 444 aa, Bacillus subtilis
MAKYTREDIEKLVKEENVKYIRLQFTDILGTIKNVEIPVSQLGKALDNKVMFDGSSIEGFVRIEESDMYLYPDLNTFVIFPWTAEKGKVARFICDIYNPDGTPFEGDPRNNLKRILKEMEDLGFSDFNLGPEPEFFLFKLDEKGEPTLELNDKGGYFDLAPTDLGENCRRDIVLELEEMGFEIEASHHEVAPGQHEIDFKYAGAVRSCDDIQTFKLVVKTIARKHGLHATFMPKPLFGVNGSGMHCNLSLFKNGVNAFFDENADLQLSETAKHFIAGIVKHATSFTAVTNPTVNSYKRLVPGYEAPCYVAWSAQNRSPLIRIPASRGISTRVEVRSVDPAANPYLALSVLLAAGLDGIKNKLEAPAPIDRNIYVMSKEERMENGIVDLPATLAEALEEFKSNEVMVKALGEHLFEHFIEAKEIEWDMFRTQVHPWEREQYMSQY

SEQ ID NO: 22 - DNA, 1335 bp, Bacillus subtilis
  source 1..1335: mol_type = genomic DNA
atggcaaagtacactagagaagatatcgaaaaattagtaaaagaagaaaacgtgaagtatatccgccttcaatttactgacattcttggaacaatcaagaatgttgagattcctgtaagccagcttggaaaagcgcttgataataaagtcatgtttgacggttcttctattgagggattcgttcgtatcgaagagtcagacatgtacctgtatccagatctaaatacatttgttatcttcccatggacagctgaaaaaggtaaagtagcacgtttcatctgtgatatttacaatccggatggcacaccttttgaaggtgacccgcgaaacaacttaaaacggattctgaaagaaatggaagacctcggcttcagtgattttaaccttgggcctgagcctgaattcttcttattcaaattggacgaaaaaggcgagccgacgcttgaactaaacgacaaaggcggatatttcgacttagctccaactgatttaggagaaaactgccgccgcgatatcgtacttgagcttgaagagatgggctttgaaatcgaagcgtctcaccacgaagtagcacctggtcagcacgaaatcgactttaaatatgctggagcagtccgctcttgtgatgacatccaaacatttaaactagttgtcaaaacaattgcccgtaaacacggcctgcatgcgacatttatgccaaaaccattgttcggtgtaaacggttcaggtatgcactgcaatctatcactcttcaaaaatggtgttaacgcattctttgacgaaaacgcagatcttcagttaagtgaaacagcgaagcacttcattgcaggtatcgtgaagcacgcaacaagctttacagcagtaacaaacccgacagtaaactcttacaaacgtcttgttcctggctatgaagcaccttgttatgtagcatggagcgcgcaaaacagaagcccgcttatccgtatcccggcttctcgcggcatcagcacacgtgttgaagtacgcagtgtagacccagctgcaaacccataccttgcacttagcgtattgcttgctgcaggattagacggaatcaaaaacaaactggaagcgccggctccaatcgaccgcaacatctatgtgatgagcaaagaagagcgcatggaaaacggaatcgttgaccttccagcaacacttgcggaagcactagaagaattcaaatcaaacgaagtcatggtcaaagcgctgggcgagcacctattcgaacacttcatcgaagcaaaagaaatcgaatgggatatgttccgcacgcaagtacatccttgggaacgcgaacagtatatgtctcagtattaa

SEQ ID NO: 23 - protein, 477 aa, Corynebacterium glutamicum
MAFETPEEIVKFIKDENVEFVDVRFTDLPGTEQHFSIPAASFDADTVEEGLAFDGSSIRGFTTIDESDMNLLPDLGTATLDPFRKAKTLNVKFFVHDPFTREAFSRDPRNVARKAEQYLASTGIADTCNFGAEAEFYLFDSVRYSTEMNSGFYEVDTEEGWWNRGKETNLDGTPNLGAKNRVKGGYFPVAPYDQTVDVRDDMVRNLAASGFALERFHHEVGGGQQEINYRFNTMLHAADDIQTFKYIIKNTARLHGKAATFMPKPLAGDNGSGMHAHQSLWKDGKPLFHDESGYAGLSDIARYYIGGILHHAGAVLAFTNATLNSYHRLVPGFEAPINLVYSQRNRSAAVRIPITGSNPKAKRIEFRAPDPSGNPYLGFAAMMMAGLDGIKNRIEPHAPVDKDLYELPPEEAASIPQAPTSLEASLKALQEDTDFLTESDVFTEDLIEAYIQYKYDNEISPVRLRPTPQEFELYFDC

SEQ ID NO: 24 - DNA, 1434 bp, Corynebacterium glutamicum
  source 1..1434: mol_type = genomic DNA
atggcgtttgaaaccccggaagaaattgtcaagttcatcaaggatgaaaacgtcgagttcgttgacgttcgattcaccgaccttcccggcaccgagcagcacttcagcatcccagctgccagcttcgatgcagatacagtcgaagaaggtctcgcattcgacggatcctcgatccgtggcttcaccacgatcgacgaatctgacatgaatctcctgccagacctcggaacggccacccttgatccattccgcaaggcaaagaccctgaacgttaagttcttcgttcacgatcctttcacccgcgaggcattctcccgcgacccacgcaacgtagcacgcaaggcagagcagtacctggcatccaccggcattgcagacacctgcaacttcggcgccgaggctgagttctacctcttcgactccgttcgctactccaccgagatgaactccggcttctacgaagtagataccgaagaaggctggtggaaccgtggcaaggaaaccaacctcgacggaaccccaaacctgggcgcaaagaaccgcgtcaagggtggctacttcccagtagcaccatacgaccaaaccgttgacgtgcgcgatgacatggttcgcaacctcgcagcttccggcttcgctcttgagcgtttccaccacgaagtcggtggcggacagcaggaaatcaactaccgcttcaacaccatgctccacgcggcagatgatatccagaccttcaagtacatcatcaagaacaccgctcgcctccacggcaaggctgcaaccttcatgcctaagccactggctggcgacaacggttccggcatgcacgctcaccagtccctctggaaggacggcaagccactcttccacgatgagtccggctacgcaggcctgtccgacatcgcccgctactacatcggcggcatcctgcaccacgcaggcgctgttctggcgttcaccaacgcaaccctgaactcctaccaccgtctggttccaggcttcgaggctccaatcaacctggtgtactcacagcgcaaccgttccgctgctgtccgtatcccaatcaccggatccaacccaaaggcaaagcgcatcgaattccgcgctccagacccatcaggcaacccatacctgggcttcgcagcgatgatgatggccggcctcgacggcatcaagaaccgcatcgagccacacgctccagtggacaaggacctctacgaactgccaccagaggaagctgcatccattccacaggcaccaacctccctggaagcatccctgaaggcactgcaggaagacaccgacttcctcaccgagtctgacgtcttcaccgaggatctcatcgaggcgtacatccagtacaagtacgacaacgagatctccccagttcgcctgcgcccaaccccgcaggaattcgaattgtacttcgactgctaa

SEQ ID NO: 25 - DNA, 39 bp, synthetic construct
  source 1..39: mol_type = other DNA
aacgacggccagtgaattcgctcgaatgcctgactgaca

SEQ ID NO: 26 - DNA, 44 bp, synthetic construct
  source 1..44: mol_type = other DNA
gtttagtactaaaccggaagggccaaaggacgacttcacggtta

SEQ ID NO: 27 - DNA, 46 bp, synthetic construct
  source 1..46: mol_type = other DNA
ccggtttagtactaaacaggaagagccattgaggatgcgaaactgt

SEQ ID NO: 28 - DNA, 39 bp, synthetic construct
  source 1..39: mol_type = other DNA
tgcatgcctgcaggtcgacgtaatcgaatcaccggccag

SEQ ID NO: 29 - DNA, 35 bp, synthetic construct
  source 1..35: mol_type = other DNA
gaaaggtgcacacatatgggttctaagtacacgag

SEQ ID NO: 30 - DNA, 37 bp, synthetic construct
  source 1..37: mol_type = other DNA
ctcttcctgtttagtttagtaaagggtaaggtactgc

SEQ ID NO: 31 - DNA, 38 bp, synthetic construct
  source 1..38: mol_type = other DNA
cccttccggtttagtgctccttagggagccatcttttg

SEQ ID NO: 32 - DNA, 35 bp, synthetic construct
  source 1..35: mol_type = other DNA
gtacttagaacccatatgtgtgcacctttcgatct

SEQ ID NO: 33 - DNA, 18 bp, synthetic construct
  source 1..18: mol_type = other DNA
tttacctcccacaagtcc

SEQ ID NO: 34 - DNA, 18 bp, synthetic construct
  source 1..18: mol_type = other DNA
aagaatctccctgccaaa

SEQ ID NO: 35 - DNA, 35 bp, synthetic construct
  source 1..35: mol_type = other DNA
aaggtgcacacatatgggtaaatacacaaaagacg

SEQ ID NO: 36 - DNA, 46 bp, synthetic construct
  source 1..46: mol_type = other DNA
ctcttcctgtttagtttaatacatttttaaatattggtcacgttcc

SEQ ID NO: 37 - DNA, 35 bp, synthetic construct
  source 1..35: mol_type = other DNA
tgtgtatttacccatatgtgtgcacctttcgatct

SEQ ID NO: 38 - DNA, 35 bp, synthetic construct
  source 1..35: mol_type = other DNA
aaaggtgcacacatatggcaaagttcacacgtgaa

SEQ ID NO: 39 - DNA, 42 bp, synthetic construct
  source 1..42: mol_type = other DNA
ctcttcctgtttagtttaatacattgacatatattgttcgcg

SEQ ID NO: 40 - DNA, 35 bp, synthetic construct
  source 1..35: mol_type = other DNA
tgtgaactttgccatatgtgtgcacctttcgatct

SEQ ID NO: 41 - DNA, 35 bp, synthetic construct
  source 1..35: mol_type = other DNA
aaggtgcacacatatgccagaatttacaagagaac

SEQ ID NO: 42 - DNA, 42 bp, synthetic construct
  source 1..42: mol_type = other DNA
ctcttcctgtttagtttagtataactctaaatattgttctct

SEQ ID NO: 43 - DNA, 35 bp, synthetic construct
  source 1..35: mol_type = other DNA
tgtaaattctggcatatgtgtgcacctttcgatct

SEQ ID NO: 44 - DNA, 35 bp, synthetic construct
  source 1..35: mol_type = other DNA
ggtgcacacatatggcaaagtatactagagaagat

SEQ ID NO: 45 - DNA, 43 bp, synthetic construct
  source 1..43: mol_type = other DNA
ctcttcctgtttagtttaaaactgagttaaatattgatcgcgt

SEQ ID NO: 46 - DNA, 35 bp, synthetic construct
  source 1..35: mol_type = other DNA
agtatactttgccatatgtgtgcacctttcgatct

SEQ ID NO: 47 - DNA, 38 bp, synthetic construct
  source 1..38: mol_type = other DNA
atgaaaaaatttacaaggaaagaaatcgaaataagtgc

SEQ ID NO: 48 - DNA, 60 bp, synthetic construct
  source 1..60: mol_type = other DNA
ctcttcctgtttagtttaatataaggttagatatttttctttttcccattcagaaacttg

SEQ ID NO: 49 - DNA, 35 bp, synthetic construct
  source 1..35: mol_type = other DNA
tgtaaattttttcatatgtgtgcacctttcgatct

SEQ ID NO: 50 - DNA, 35 bp, synthetic construct
  source 1..35: mol_type = other DNA
atgaaaaattttactagagaagaaatcgtaacaag

SEQ ID NO: 51 - DNA, 47 bp, synthetic construct
  source 1..47: mol_type = other DNA
ctcttcctgtttagtttaataaagagtcatatacttttcttgttccc

SEQ ID NO: 52 - DNA, 35 bp, synthetic construct
  source 1..35: mol_type = other DNA
agtaaaatttttcatatgtgtgcacctttcgatct

SEQ ID NO: 53 - DNA, 35 bp, synthetic construct
  source 1..35: mol_type = other DNA
gaaaggtgcacacatatggcaaaacagtcctattc

SEQ ID NO: 54 - DNA, 43 bp, synthetic construct
  source 1..43: mol_type = other DNA
ctcttcctgtttagtttaatacagttccatgtactgatcacgt

SEQ ID NO: 55 - DNA, 35 bp, synthetic construct
  source 1..35: mol_type = other DNA
ggactgttttgccatatgtgtgcacctttcgatct

SEQ ID NO: 56 - DNA, 35 bp, synthetic construct
  source 1..35: mol_type = other DNA
aaggtgcacacatatgccaggacttccaaaaaatg

SEQ ID NO: 57 - DNA, 54 bp, synthetic construct
  source 1..54: mol_type = other DNA
ctcttcctgtttagtttaagaatctagatactgatatatttccataggatgtgg

SEQ ID NO: 58 - DNA, 35 bp, synthetic construct
  source 1..35: mol_type = other DNA
tggaagtcctggcatatgtgtgcacctttcgatct

SEQ ID NO: 59 - DNA, 35 bp, synthetic construct
  source 1..35: mol_type = other DNA
gaaaggtgcacacatatgcctaactataccaggga

SEQ ID NO: 60 - DNA, 40 bp, synthetic construct
  source 1..40: mol_type = other DNA
ctcttcctgtttagtttaatatctggtgagatactggtcg

SEQ ID NO: 61 - DNA, 35 bp, synthetic construct
  source 1..35: mol_type = other DNA
ggtatagttaggcatatgtgtgcacctttcgatct

SEQ ID NO: 62 - DNA, 37 bp, synthetic construct
  source 1..37: mol_type = other DNA
gaaaggtgcacacatatggcaaagtacactagagaag

SEQ ID NO: 63 - DNA, 40 bp, synthetic construct
  source 1..40: mol_type = other DNA
ctcttcctgtttagtttaatactgagacatatactgttcg

SEQ ID NO: 64 - DNA, 36 bp, synthetic construct
  source 1..36: mol_type = other DNA
agtgtactttgccatatgtgtgcacctttcgatcta

SEQ ID NO: 65 - DNA, 35 bp, synthetic construct
  source 1..35: mol_type = other DNA
gaaaggtgcacacatatggcgtttgaaaccccgga

SEQ ID NO: 66 - DNA, 39 bp, synthetic construct
  source 1..39: mol_type = other DNA
ctcttcctgtttagtttagcagtcgaagtacaattcgaa

SEQ ID NO: 67 - DNA, 38 bp, synthetic construct
  source 1..38: mol_type = other DNA
ggtttcaaacgccatatgtgtgcacctttcgatctacg